European Patent Application EP 4 545 570 A1, published April 30, 2025. Title: Fusion Proteins Comprising an Improved GLP-1 Receptor Agonist and Uses Thereof. Applicant: Guangzhou Innogen Pharmaceutical Group Co., Ltd.; Shanghai Innogen Pharmaceutical Technology Co., Ltd.; Shanghai Innogen Biomedical Engineering Co., Ltd. The sequence listing filed with the application follows.

SEQUENCE LISTING (43 sequences)

SEQ ID NO: 1 - protein, 30 aa, synthetic construct
HAEGTFTSDVSSYLEGQAAKEFIAWLVKGR

SEQ ID NO: 2 - protein, 31 aa, synthetic construct
HAEGTFTSDVSSYLEGQAAKEFIAWLVKGRG

SEQ ID NO: 3 - protein, 31 aa, synthetic construct
HGEGTFTSDVSSYLEEQAAKEFIAWLVKGGG

SEQ ID NO: 4 - protein, 16 aa, synthetic construct
MPLLLLLPLLWAGALA

SEQ ID NO: 5 - protein, 227 aa, synthetic construct
ERKCCVECPPCPAPPVAGPSVFLFPPKPKDTLMISRTPEVTCVVVDVSHEDPEVQFNWYVDGVEVHNAKTKPREEQFNSTFRVVSVLTVVHQDWLNGKEYKCKVSNKGLPAPIEKTISKTKGQPREPQVYTLPPSREEMTKNQVSLTCLVKGFYPSDIAVEWESNGQPENNYKTTPPMLDSDGSFFLYSKLTVDKSRWQQGNVFSCSVMHEALHNHYTQKSLSLSPG

SEQ ID NO: 6 - protein, 227 aa, synthetic construct
ERKSCVECPPCPAPPVAGPSVFLFPPKPKDTLMISRTPEVTCVVVDVSHEDPEVQFNWYVDGVEVHNAKTKPREEQFNSTFRVVSVLTVVHQDWLNGKEYKCKVSNKGLPSSIEKTISKTKGQPREPQVYTLPPSREEMTKNQVSLTCLVKGFYPSDIAVEWESNGQPENNYKTTPPMLDSDGSFFLYSKLTVDKSRWQQGNVFSCSVMHEALHNHYTQKSLSLSPG

SEQ ID NO: 7 - protein, 271 aa, synthetic construct
HGEGTFTSDVSSYLEEQAAKEFIAWLVKGGGSSGAPPPSGGGGSERKSCVECPPCPAPPVAGPSVFLFPPKPKDTLMISRTPEVTCVVVDVSHEDPEVQFNWYVDGVEVHNAKTKPREEQFNSTFRVVSVLTVVHQDWLNGKEYKCKVSNKGLPSSIEKTISKTKGQPREPQVYTLPPSREEMTKNQVSLTCLVKGFYPSDIAVEWESNGQPENNYKTTPPMLDSDGSFFLYSKLTVDKSRWQQGNVFSCSVMHEALHNHYTQKSLSLSPG

SEQ ID NO: 8 - protein, 287 aa, synthetic construct
MPLLLLLPLLWAGALAHGEGTFTSDVSSYLEEQAAKEFIAWLVKGGGSSGAPPPSGGGGSERKSCVECPPCPAPPVAGPSVFLFPPKPKDTLMISRTPEVTCVVVDVSHEDPEVQFNWYVDGVEVHNAKTKPREEQFNSTFRVVSVLTVVHQDWLNGKEYKCKVSNKGLPSSIEKTISKTKGQPREPQVYTLPPSREEMTKNQVSLTCLVKGFYPSDIAVEWESNGQPENNYKTTPPMLDSDGSFFLYSKLTVDKSRWQQGNVFSCSVMHEALHNHYTQKSLSLSPG

SEQ ID NO: 9 - protein, 13 aa, synthetic construct
SSGAPPPSGGGGS

SEQ ID NO: 10 - protein, 15 aa, synthetic construct
GGGGSGGGGSGGGGS

SEQ ID NO: 11 - protein, 20 aa, synthetic construct
GGGGSGGGGSGGGGSGGGGS

SEQ ID NO: 12 - protein, 20 aa, synthetic construct
GSTGGGGSGKPGSGEGGGGS

SEQ ID NO: 13 - protein, 15 aa, synthetic construct
ESGRSGGGGSGGGGS

SEQ ID NO: 14 - protein, 14 aa, synthetic construct
EGKSSGSGSESKST

SEQ ID NO: 15 - protein, 15 aa, synthetic construct
EGKSSGSGSESKSTQ

SEQ ID NO: 16 - protein, 14 aa, synthetic construct
EGKSSGSGSESKVD

SEQ ID NO: 17 - protein, 14 aa, synthetic construct
GSTSGSGKSSEGKG

SEQ ID NO: 18 - protein, 18 aa, synthetic construct
KESGSVSSEQLAQFRSLD

SEQ ID NO: 19 - protein, 16 aa, synthetic construct
ESGSVSSEELAFRSLD

SEQ ID NO: 20 - protein, 90 aa, synthetic construct
CACGCCGAGGGCACCTTCACCAGCGACGTGAGCAGCTACCTGGAGGGCCAGGCCGCCAAGGAGTTCATCGCCTGGCTGGTGAAGGGCAGG

SEQ ID NO: 21 - protein, 93 aa, synthetic construct
CACGCCGAGGGCACCTTCACCAGCGACGTGAGCAGCTACCTGGAGGGCCAGGCCGCCAAGGAGTTCATCGCCTGGCTGGTGAAGGGCAGGGGC

SEQ ID NO: 22 - protein, 93 aa, synthetic construct
CACGGCGAGGGCACCTTCACCAGCGACGTGAGCAGCTACCTGGAGGAGCAGGCCGCCAAGGAGTTCATCGCCTGGCTGGTGAAGGGCGGCGGC

SEQ ID NO: 23 - protein, 48 aa, synthetic construct
ATGCCCCTGCTGCTGCTGCTGCCCCTGCTGTGGGCCGGCGCCCTGGCC

SEQ ID NO: 24 - protein, 681 aa, synthetic construct
GAGAGGAAGTGCTGCGTGGAGTGCCCCCCCTGCCCCGCCCCCCCCGTGGCCGGCCCCAGCGTGTTCCTGTTCCCCCCCAAGCCCAAGGACACCCTGATGATCAGCAGGACCCCCGAGGTGACCTGCGTGGTGGTGGACGTGAGCCACGAGGACCCCGAGGTGCAGTTCAACTGGTACGTGGACGGCGTGGAGGTGCACAACGCCAAGACCAAGCCCAGGGAGGAGCAGTTCAACAGCACCTTCAGGGTGGTGAGCGTGCTGACCGTGGTGCACCAGGACTGGCTGAACGGCAAGGAGTACAAGTGCAAGGTGAGCAACAAGGGCCTGCCCGCCCCCATCGAGAAGACCATCAGCAAGACCAAGGGCCAGCCCAGGGAGCCCCAGGTGTACACCCTGCCCCCCAGCAGGGAGGAGATGACCAAGAACCAGGTGAGCCTGACCTGCCTGGTGAAGGGCTTCTACCCCAGCGACATCGCCGTGGAGTGGGAGAGCAACGGCCAGCCCGAGAACAACTACAAGACCACCCCCCCCATGCTGGACAGCGACGGCAGCTTCTTCCTGTACAGCAAGCTGACCGTGGACAAGAGCAGGTGGCAGCAGGGCAACGTGTTCAGCTGCAGCGTGATGCACGAGGCCCTGCACAACCACTACACCCAGAAGAGCCTGAGCCTGAGCCCCGGC

SEQ ID NO: 25 - protein, 681 aa, synthetic construct
GAGAGGAAGAGCTGCGTGGAGTGCCCCCCCTGCCCCGCCCCCCCCGTGGCCGGCCCCAGCGTGTTCCTGTTCCCCCCCAAGCCCAAGGACACCCTGATGATCAGCAGGACCCCCGAGGTGACCTGCGTGGTGGTGGACGTGAGCCACGAGGACCCCGAGGTGCAGTTCAACTGGTACGTGGACGGCGTGGAGGTGCACAACGCCAAGACCAAGCCCAGGGAGGAGCAGTTCAACAGCACCTTCAGGGTGGTGAGCGTGCTGACCGTGGTGCACCAGGACTGGCTGAACGGCAAGGAGTACAAGTGCAAGGTGAGCAACAAGGGCCTGCCCAGCAGCATCGAGAAGACCATCAGCAAGACCAAGGGCCAGCCCAGGGAGCCCCAGGTGTACACCCTGCCCCCCAGCAGGGAGGAGATGACCAAGAACCAGGTGAGCCTGACCTGCCTGGTGAAGGGCTTCTACCCCAGCGACATCGCCGTGGAGTGGGAGAGCAACGGCCAGCCCGAGAACAACTACAAGACCACCCCCCCCATGCTGGACAGCGACGGCAGCTTCTTCCTGTACAGCAAGCTGACCGTGGACAAGAGCAGGTGGCAGCAGGGCAACGTGTTCAGCTGCAGCGTGATGCACGAGGCCCTGCACAACCACTACACCCAGAAGAGCCTGAGCCTGAGCCCCGGC

SEQ ID NO: 26 - protein, 813 aa, synthetic construct
CACGGCGAGGGCACCTTCACCAGCGACGTGAGCAGCTACCTGGAGGAGCAGGCCGCCAAGGAGTTCATCGCCTGGCTGGTGAAGGGCGGCGGCAGCAGCGGCGCCCCCCCCCCCAGCGGCGGCGGCGGCAGCGAGAGGAAGAGCTGCGTGGAGTGCCCCCCCTGCCCCGCCCCCCCCGTGGCCGGCCCCAGCGTGTTCCTGTTCCCCCCCAAGCCCAAGGACACCCTGATGATCAGCAGGACCCCCGAGGTGACCTGCGTGGTGGTGGACGTGAGCCACGAGGACCCCGAGGTGCAGTTCAACTGGTACGTGGACGGCGTGGAGGTGCACAACGCCAAGACCAAGCCCAGGGAGGAGCAGTTCAACAGCACCTTCAGGGTGGTGAGCGTGCTGACCGTGGTGCACCAGGACTGGCTGAACGGCAAGGAGTACAAGTGCAAGGTGAGCAACAAGGGCCTGCCCAGCAGCATCGAGAAGACCATCAGCAAGACCAAGGGCCAGCCCAGGGAGCCCCAGGTGTACACCCTGCCCCCCAGCAGGGAGGAGATGACCAAGAACCAGGTGAGCCTGACCTGCCTGGTGAAGGGCTTCTACCCCAGCGACATCGCCGTGGAGTGGGAGAGCAACGGCCAGCCCGAGAACAACTACAAGACCACCCCCCCCATGCTGGACAGCGACGGCAGCTTCTTCCTGTACAGCAAGCTGACCGTGGACAAGAGCAGGTGGCAGCAGGGCAACGTGTTCAGCTGCAGCGTGATGCACGAGGCCCTGCACAACCACTACACCCAGAAGAGCCTGAGCCTGAGCCCCGGC

SEQ ID NO: 27 - protein, 861 aa, synthetic construct
ATGCCCCTGCTGCTGCTGCTGCCCCTGCTGTGGGCCGGCGCCCTGGCCCACGGCGAGGGCACCTTCACCAGCGACGTGAGCAGCTACCTGGAGGAGCAGGCCGCCAAGGAGTTCATCGCCTGGCTGGTGAAGGGCGGCGGCAGCAGCGGCGCCCCCCCCCCCAGCGGCGGCGGCGGCAGCGAGAGGAAGAGCTGCGTGGAGTGCCCCCCCTGCCCCGCCCCCCCCGTGGCCGGCCCCAGCGTGTTCCTGTTCCCCCCCAAGCCCAAGGACACCCTGATGATCAGCAGGACCCCCGAGGTGACCTGCGTGGTGGTGGACGTGAGCCACGAGGACCCCGAGGTGCAGTTCAACTGGTACGTGGACGGCGTGGAGGTGCACAACGCCAAGACCAAGCCCAGGGAGGAGCAGTTCAACAGCACCTTCAGGGTGGTGAGCGTGCTGACCGTGGTGCACCAGGACTGGCTGAACGGCAAGGAGTACAAGTGCAAGGTGAGCAACAAGGGCCTGCCCAGCAGCATCGAGAAGACCATCAGCAAGACCAAGGGCCAGCCCAGGGAGCCCCAGGTGTACACCCTGCCCCCCAGCAGGGAGGAGATGACCAAGAACCAGGTGAGCCTGACCTGCCTGGTGAAGGGCTTCTACCCCAGCGACATCGCCGTGGAGTGGGAGAGCAACGGCCAGCCCGAGAACAACTACAAGACCACCCCCCCCATGCTGGACAGCGACGGCAGCTTCTTCCTGTACAGCAAGCTGACCGTGGACAAGAGCAGGTGGCAGCAGGGCAACGTGTTCAGCTGCAGCGTGATGCACGAGGCCCTGCACAACCACTACACCCAGAAGAGCCTGAGCCTGAGCCCCGGC

SEQ ID NO: 28 - protein, 39 aa, synthetic construct
AGCAGCGGCGCCCCCCCCCCCAGCGGCGGCGGCGGCAGC

SEQ ID NO: 29 - protein, 45 aa, synthetic construct
GGCGGCGGCGGCAGCGGCGGCGGCGGCAGCGGCGGCGGCGGCAGC

SEQ ID NO: 30 - protein, 60 aa, synthetic construct
GGCGGCGGCGGCAGCGGCGGCGGCGGCAGCGGCGGCGGCGGCAGCGGCGGCGGCGGCAGC

SEQ ID NO: 31 - protein, 60 aa, synthetic construct
GGCAGCACCGGCGGCGGCGGCAGCGGCAAGCCCGGCAGCGGCGAGGGCGGCGGCGGCAGC

SEQ ID NO: 32 - protein, 45 aa, synthetic construct
GAGAGCGGCAGGAGCGGCGGCGGCGGCAGCGGCGGCGGCGGCAGC

SEQ ID NO: 33 - protein, 42 aa, synthetic construct
GAGGGCAAGAGCAGCGGCAGCGGCAGCGAGAGCAAGAGCACC

SEQ ID NO: 34 - protein, 45 aa, synthetic construct
GAGGGCAAGAGCAGCGGCAGCGGCAGCGAGAGCAAGAGCACCCAG

SEQ ID NO: 35 - protein, 42 aa, synthetic construct
GAGGGCAAGAGCAGCGGCAGCGGCAGCGAGAGCAAGGTGGAC

SEQ ID NO: 36 - protein, 42 aa, synthetic construct
GGCAGCACCAGCGGCAGCGGCAAGAGCAGCGAGGGCAAGGGC

SEQ ID NO: 37 - protein, 54 aa, synthetic construct
AAGGAGAGCGGCAGCGTGAGCAGCGAGCAGCTGGCCCAGTTCAGGAGCCTGGAC

SEQ ID NO: 38 - protein, 48 aa, synthetic construct
GAGAGCGGCAGCGTGAGCAGCGAGGAGCTGGCCTTCAGGAGCCTGGAC

SEQ ID NO: 39 - protein, 4 aa, synthetic construct
GGGS

SEQ ID NO: 40 - protein, 5 aa, synthetic construct
GGGGS

SEQ ID NO: 41 - protein, 6 aa, synthetic construct
GGGGGS

SEQ ID NO: 42 - protein, 8 aa, synthetic construct
GGGGGGGS

SEQ ID NO: 43 - protein, 37 aa, synthetic construct
HDEFERHAEGTFTSDVSSYLEGQAAKEFIAWLVKGRG